European Patent Application EP 4 442 817 A1, published October 9, 2024. Title: Paclitaxel (taxol) biosynthesis pathway. Applicant: Max-Planck-Gesellschaft zur Förderung der Wissenschaften e.V. Application EP. The sequence listing filed with the application follows.

SEQUENCE LISTING (48 sequences)

SEQ ID NO: 1 - protein, 862 aa, Taxus baccata
  source 1..862: note = taxadiene synthase
MAQLSFNAALKMNALGNKAIHDPTNCRAKSEGQMMWVCSKSGRTRVKMSRGSGGPGPVVMMSSSTGTSKVVSETSSTIVDDIPRLSANYHGDLWHHNVIQTLETPFRESSTYQERADELVVKIKDMFNALGDGDISPSAYDTAWVARVATISSDGSEKPRFPQALNWVFNNQLQDGSWGIESHFSLCDRLLNTTNSVIALSVWKTGHSQVEQGTEFIAENLRLLNEEDELSPDFEIIFPALLQKAKALGINLPYDLPFIKSLSTTREARLTDVSAAADNIPANMLNALEGLEEVIDWNKIMRFQSKDGSFLSSPASTACVLMNIGDEKCFTFLNNLLDKFGGCVPCMYSIDLLERLSLVDNIEHLGIGRHFKQEIKGALDYVYRHWSERGIGWGRDSLVPDLNTTALGLRTLRTHGYDVSSDVLNNFKDENGRFFSSAGQTHVELRSVVNLFRASDLAFPDEGVMDDARKFAEPYLRDALATKISTNTKLFKEIEYVVEYPWHMSIPRLEAGSYIDSYDDDYVWQRKTLYRMPSLSNSKCLELAKLDFNIVQSLHQEELKLLTRWWKESGMADINFTRHRVAEVYFSSATFEPEYSATRIAFTKIGCLQVLFDDMADIFATLDELKSFTEGVKRWDTSLLHEIPECMQTCFKVWFKLMEEVNNDVVKVQGRDMLAHIRKPWELYFNCYVQEREWLEAGYIPTFEEYLKTYAISVGLGPCTLQPILLMGELVKDDVVEKVHYPSNMFELVSLSWRLTNDTKTYQAEKARGQQASGIACYMKDNPGATEEDAIKHICRVVDRALKEASFEYFKPSNDIPMGCKSFIFNLRLCVQIFYKFIDGYGIANEEIKDYIRKVYIDPIQV

SEQ ID NO: 2 - RNA, 2589 nt, Taxus baccata
  source 1..2589: mol_type = mRNA; note = taxadiene synthase
atggctcagctctcatttaatgcagcgctgaagatgaatgcattagggaacaaggcaatccacgatccaacgaattgcagagccaaatctgagggccaaatgatgtgggtttgctccaaatcagggcgaaccagagtaaaaatgtcgagaggaagtggtggtcctggtcctgtcgtaatgatgagcagtagcactggcactagcaaggtggtttccgagacttccagtaccattgtggatgatatccctcgactctccgccaattatcatggcgatctgtggcaccacaatgttatacaaactctggagacaccatttcgtgagagttctacttaccaagaacgggcagatgagctggttgtgaaaattaaagatatgttcaatgcgctcggagacggagatatcagtccgtctgcatacgacactgcgtgggtggcgagggtggcgaccatttcctctgatggatctgagaagccacggtttcctcaggccctcaactgggttttcaacaaccagctccaggatggatcgtggggtatcgaatcgcactttagtttatgcgatcgattgcttaacacgaccaattctgttatcgccctctcggtttggaaaacagggcacagccaagtagaacaaggtactgagtttattgcagagaatctaagattactcaatgaggaagatgagctgtccccggatttcgaaataatctttcctgctctgctgcaaaaggcaaaagcgttggggatcaatcttccttacgatcttccatttatcaaatctttgtcgacaacacgggaagccaggcttacagatgtttctgcggcagcagacaatattccagccaacatgttgaatgcgttggagggtctcgaggaagttattgactggaacaagattatgaggtttcaaagtaaagatggatctttcctgagctcccctgcctccactgcctgtgtactgatgaatataggggacgaaaaatgtttcacttttctcaacaatctgctggacaaattcggcggctgcgtgccctgtatgtattccatcgatctgctggaacgcctttcgctggttgataacattgagcatctcggaatcggtcgccatttcaaacaagaaatcaaaggagctcttgattatgtctacagacattggagtgaaaggggcatcggttggggcagagacagcctcgttccagatctcaacacaacagccctcggcctgcgaactcttcgcacgcacggatacgatgtttcttcagatgttttgaataatttcaaagatgaaaacgggcggttcttctcctctgcgggccaaacccatgtcgaattgagaagcgtggtgaatcttttcagagcttccgaccttgcatttcctgacgaaggagttatggacgatgctagaaaatttgcagaaccatatcttagagacgcacttgcaacaaaaatctcaaccaatacaaaactattcaaagagattgagtacgtggtggagtacccttggcacatgagtatcccacgtctagaagccggaagttatattgattcatatgacgatgattatgtatggcagaggaagactctatacagaatgccatctttgagtaattcaaaatgtttagaattggcaaaattggacttcaatatcgtacaatctttgcatcaagaggagttgaagcttctaacaagatggtggaaggaatctggcatggcagatataaatttcactcgacaccgagtggcggaggtttatttttcatcagctacatttgaacccgaatattctgccactcgaattgccttcacaaaaattggttgtttacaagtcctttttgatgatatggctgacatctttgcaacactagatgaattgaaaagtttcactgagggagtaaagagatgggatacatctttgctacatgagattccagagtgtatgcaaacttgctttaaagtttggttcaaattgatggaagaagtaaataatgatgtggttaaggtacaaggacgtgacatgctcgctcacataagaaaaccctgggagttgtacttcaattgttatgtacaagaaagggagtggcttgaagctgggtatataccaacttttgaagagtacttaaagacttatgctatatcagtaggccttggaccgtgtaccctacaaccaatactactaatgggtgagcttgtgaaagatgatgttgttgagaaagtgcactatccctcaaatatgtttgagcttgtatccttgagctggcgactaacaaatgacaccaaaacatatcaggctgaaaaggctcgaggacaacaagcctcaggcatagcatgctatatgaaggataatccaggagcaactgaggaagatgccatcaagcacatatgtcgtgttgttgaccgagccttgaaagaagcaagctttgaatatttcaaaccatccaatgatatcccaatgggttgcaagtcctttatttttaaccttagattgtgtgtccaaatcttttacaagtttatagatgggtacggaatcgccaatgaggagattaaggattatataagaaaagtttatattgatccaattcaagtatga

SEQ ID NO: 3 - protein, 274 aa, Taxus baccata
  source 1..274: note = C4 beta, C20-epoxidase
MTEIDLPGIDISQFPPEIAGDHFQYHADLAKLREACKEWGFFRVVNHGIPPDLIEKVVSVTQDLLSMPVELKDTVTTSNPMESYLRFPNFEVFYLVGMPNPRSIQEICEKIWPQGNSNFCEAVGKFTLLQSNLATKIIKIILASLGLDARKFYQSDFKKCSAKFHINGYPSHGKRMGDVVLPCHGDVNCMTILYNDENAGLQVRSKEGEWFNVKPQPDSFVVNIGDCLRAWSNGRYRSADHRVIYTGWKHRISLPYSINFPHHFQIYAPQELVG

SEQ ID NO: 4 - RNA, 825 nt, Taxus baccata
  source 1..825: mol_type = mRNA; note = C4 beta, C20-epoxidase
atgactgaaattgaccttcccgggattgacatttcacaatttcctcccgaaatcgcgggagatcattttcagtatcatgcagatctagcgaagctcagagaagcatgcaaagaatgggggtttttccgcgtcgtgaatcatgggattccacccgatcttattgagaaggttgtgtctgtaacccaagatttattgtcgatgcccgtggagttgaaggacacagtcacaacttctaatcccatggaaagttacttacgctttccaaactttgaggtgttctacctcgtgggcatgcccaatccgcgttcaattcaggaaatttgtgaaaagatatggccccaagggaactcaaatttctgcgaagcggttggcaaatttaccttacttcagtcaaatctggcgactaagatcattaaaatcattcttgcaagccttggtttggatgcgaggaaattctaccaatctgatttcaaaaaatgctcagccaaatttcatataaacggttatccatctcatggaaaacgtatgggggacgtggttttgccttgtcacggagatgtaaactgtatgactatcctttacaacgatgaaaatgcaggtctccaggttcgatccaaagaaggagagtggttcaacgtcaaacctcaaccagattcattcgttgtcaacattggggattgcctaagggcatggagcaatggtaggtaccgcagcgcagatcaccgcgttatctacacagggtggaagcatcgtatatctcttccctattcaataaacttcccgcaccatttccaaatttatgctcctcaggagcttgtnggatga

SEQ ID NO: 5 - protein, 499 aa, Taxus baccata
  source 1..499: note = taxane 5 alpha-hydroxylase
MDALYKSTVAKFNEVTQLDCSTESFSIALSAIAGILLLLLLFRSKRHSSLKLPPGKLGIPFIGESFIFLRALRSNSLEQFFDERVKKFGLVFKTSLIGHPTVVLCGPAGNRLILSNEEKLVQMSWPAQFMKLMGENSVATRRGEDHIVMRSALAGFFGPGALQSYIGKMNTEIQSHINEKWKGKDEVNVLPLVRELVFNISAILFFNIYDKQEQDRLHKLLETILVGSFALPIDLPGFGFHRALQGRAKLNKIMLSLIKKRKEDLQSGSATATQDLLSVLLTFRDDKGTPLTNDEILDNFSSLLHASYDTTTSPMALIFKLLSSNPECYQKVVQEQLEILSNKEEGEEITWKDLKAMKYTWQVAQETLRMFPPVFGTFRKAITDIQYDGYTIPKGWKLLWTTYSTHPKDLYFNEPEKFMPSRFDQEGKHVAPYTFLPFGGGQRSCVGWEFSKMEILLFVHHFVKTFSSYTPVDPDEKISGDPLPPLPSKGFSIKLFPRP

SEQ ID NO: 6 - RNA, 1500 nt, Taxus baccata
  source 1..1500: mol_type = mRNA; note = taxane 5 alpha-hydroxylase
atggacgccctgtataagagcacagttgcaaaatttaatgaggtcacacagctggactgttccactgaatctttttccattgccctctcagctattgctggtattcttctgcttctcctgctcttccgttctaaacgccactcctcccttaaacttcctcctgggaaattaggcatccctttcattggcgagtcgtttatcttcctgagggctcttcgatcgaactcgctggagcaattttttgacgagagagtgaagaaattcggcctcgtgttcaagacctccttgattgggcatcccacagtagtactctgcggccctgcgggaaaccggcttattctgtccaacgaggagaagctggtgcagatgtcgtggcccgctcaatttatgaagctcatgggggagaattccgttgccaccaggaggggtgaagaccatatagttatgcgctctgctcttgcaggttttttcggccctggtgcgctgcagagttacattggtaaaatgaatacagagatccagagtcatatcaacgaaaaatggaagggaaaagatgaggtgaatgtacttcctttggtaagagagctcgtcttcaacatttcggccatcttgtttttcaacatatatgataagcaggaacaggatcgtctgcataagcttttggaaactattctggtcggaagttttgctcttccgattgacttgcccggatttggtttccatagagcactccagggacgggccaagctcaacaaaattatgctgtctttaattaaaaagagaaaagaagatctgcagtctggatcggcaacagccacgcaggatctgctctctgttttgctcactttcagagatgacaaagggactccactcaccaatgatgagatactcgacaacttttcttctctgctccatgcctcctatgacaccaccacttcgccaatggctttgattttcaagctcttgtcttccaatccagaatgctatcaaaaagtagttcaagagcaattggagatactttccaacaaagaggagggcgaagaaatcacatggaaggatctcaaagccatgaaatacacatggcaagtagctcaggaaacgctgcggatgtttcctccagttttcggaacatttcgcaaggccatcactgacattcagtatgatggttacacaattccaaaagggtggaagctgttgtggacaacttacagtacacatcccaaggacttgtatttcaatgaaccagagaaattcatgccttcaagattcgatcaggaaggaaagcatgtagctccttacacatttttgcccttcggtggaggccaacggtcatgtgtgggatgggaattttcaaagatggagatattactattcgttcatcattttgtcaaaacttttagcagctacaccccagttgatcccgacgaaaaaatatcaggggatccactccctcctcttccttccaagggattttccattaaactgtttccgagaccatag

SEQ ID NO: 7 - protein, 495 aa, Taxus baccata
  source 1..495: note = taxane 2 alpha-hydroxylase
MDAMDLTVAKFKEFTQLQSSAILLTVVSGIIVIVILLLRSKRRSSLKLPPGKLGLPLIGESLSFLWALRSNTLEQFVDKRVKKYGNVFKTSLLGQPTVVLCGAAGNRLILSNQEKLLSRTVSDRVAKLTGDTSISVIAGDSHRIIRAAVAGFLGPAGLKIHIGEMSAHIRNHINQVWKGKDEVNVLSLARELVFAISASLFLNINDREEQHQLHKTLETILPGYFSVPINFPGFAFRKALEGNSKRRKHFSVLQEKRRRDLSVGLASRTQDLLSVLLAYEDDKGNPLTDEEVLDNISALIDGSYESTSSQMAMLLKLLSDHPECYEKVVQEQLEIASHKKEGEEITWKDVKAMRYTWQVMQETLRMFAPVFGPRGKAITDIHYDGYTIPKGWQLSWATYSTHQNDTYFNEPDKFMPSRFDEEGGRLAPYTFVPFGGGRRKCPGWEFAKTEILLFVHHFVKTFSAYTPIDPHESIWGRPLPPVPANGFPIKLISRS

SEQ ID NO: 8 - RNA, 1488 nt, Taxus baccata
  source 1..1488: mol_type = mRNA; note = taxane 2 alpha-hydroxylase
atggacgccatggatctcacagttgcaaagtttaaggaattcacgcagctacagtcctctgctattcttctcactgttgtttctggaatcatcgtcatcgtaatcctgctcctccgttctaaacgccgctcctctctcaaacttcctccggggaaattaggcctccctctcattggggaatcgttatcattcctgtgggctcttcgatcaaacacactcgaacagtttgtggacaaaagagtgaagaaatacggcaatgtcttcaagacatcgttacttgggcaacccacagtagtactgtgtggcgcagccggaaaccgcctaattctgtcgaaccaggagaagctgttgagccgaacggtgtcggatcgagtagcgaaactgacgggtgatacttctatttcggttatagcgggagacagtcatcgcatcatacgcgcagcagttgcagggtttttggggccagcaggactcaagattcacattggcgaaatgagcgcacatatccgaaatcatatcaaccaagtatggaagggaaaagatgaagtgaacgtacttagtttggcaagagagctggtcttcgccatctcggccagtttgtttttaaatataaatgatagagaggaacagcaccaattgcataagactctcgaaactattcttcccggatatttttctgttcctataaacttccccggatttgcctttcgcaaggcactggagggaaactcgaagcgtaggaaacatttctctgttttacaagaaaagagaagaagggatctgagcgtagggttagcatcccgcactcaggatctgctttctgttttgctcgcctacgaagatgacaaagggaatccactcaccgatgaggaggtcctcgacaacatttctgcgctcattgatggctcctacgagagcacctcttcacaaatggccatgcttttaaagctgttgtctgaccatccagaatgctatgaaaaagtagttcaagagcaattggagatagcttcacataaaaaggaaggagaagaaatcacatggaaggatgtgaaagccatgagatacacatggcaagtaatgcaggagacgctgcggatgtttgcccctgtttttggacctcgtgggaaagctataactgacattcattatgacggttacaccattccaaaaggatggcaactttcatgggcaacttattcgacccatcagaatgatacatatttcaatgagccggacaaattcatgccgtccagattcgacgaggaaggagggcgtttggctccttacacattcgtgccatttggaggagggagaaggaaatgcccaggatgggaattcgcaaagactgagatattactgttcgtccatcattttgttaaaacattcagtgcctacacgccaatcgaccctcacgaaagtatttgggggcgtccactccctcctgtccctgccaatggatttcctattaaacttatttctcgatcctaa

SEQ ID NO: 9 - protein, 500 aa, Taxus baccata
  source 1..500: note = taxane 7 beta-hydroxylase
MDALSLVNSTVAKFNEVTQLQASPAILSTALTAIAGIIVLLVITSKRRSSLKLPPGKLGLPFIGETLEFVKALRSDTLRQFVEEREGKFGRVFKTSLLGKPTVILCGPAGNRLVLSNEEKLLHVSWSAQIARILGLNSVAVKRGDDHRVLRVALAGFLGSAGLQLYIGKMSALIRNHINEKWKGKDEVNVLSLVRDLVMDNSAILFFNIYDKERKQQLHEILKIILASHFGIPLNIPGFLYRKALKGSLKRKKILSALLEKRKDELRSRLASSNQDLLSVLLSFRDERGKPLSDEAVLDNCFAMLDASYDTTTSQMTLILKMLSSNPECFEKVVQEQLEIASNKKEGEEITMKDIKAMKYTWQVLQESLRMLSPVFGTLRKTMNDINHDGYTIPKGWQVVWTTYSTHQKDIYFKQPDKFMPSRFEEEDGHLDAYTFVPFGGGRRTCPGWEYAKVEILLFLHHFVKAFSGYTPTDPHERICGYPVPLVPVKGFPIKLIARS

SEQ ID NO: 10 - RNA, 1503 nt, Taxus baccata
  source 1..1503: mol_type = mRNA; note = taxane 7 beta-hydroxylase
atggatgccctttctcttgtaaacagcacagttgcaaaatttaatgaggtaacgcagctacaggcttcccctgctattctgtccactgccctcactgctattgcaggcattattgtgctcctcgtcatcacttctaaacgccgttcctctcttaaacttcctcctggaaaactaggcctccctttcattggcgagactttagagttcgtgaaggctcttcgatcagacacacttcgacaatttgtggaggaaagggaggggaaatttggacgtgtgttcaagacttcattgcttgggaagcccactgtaatactctgcggccctgcgggaaaccgcttagttctttccaacgaggaaaaactgttgcacgtgtcgtggtccgcccaaattgccagaatcctgggtctcaattctgttgcagtgaaaaggggagatgatcaccgcgttctgcgtgtcgcactagcaggttttttgggctctgcagggctacagctttacataggtaaaatgagtgcacttatcagaaatcatatcaatgaaaaatggaagggaaaagatgaagtgaatgtactgagtttggtaagagatcttgtcatggacaattcagctatcttgtttttcaatatatacgataaagagcgaaagcaacaactgcatgaaatattgaaaatcattcttgcctcacatttcggcatacctttaaacattcccggatttctgtatcgcaaagcactcaaggggagcttgaagcggaaaaaaattctctccgctttactggaaaagagaaaagacgaactgcgctcaagattagcgtctagcaatcaagatcttctctctgttttgctcagcttcagagatgaaagagggaaaccactgagcgacgaggcagtcttagacaactgttttgcaatgctggatgcctcctatgacaccaccacttcacaaatgactctgattttaaagatgttgtcttccaatccagaatgctttgaaaaagtagttcaagagcaattggagatagcgtcaaataaaaaggagggagaagaaatcacaatgaaggatatcaaagccatgaaatacacatggcaagtgctccaggaaagtctacggatgctttctccagtatttggaacacttcgtaagaccatgaatgacattaatcacgatggttacacaattccaaaaggatggcaggttgtatggacaacttattctacacatcagaaagacatatatttcaagcagccagataaattcatgccttcgagattcgaagaggaagatgggcatttggatgcttatacattcgtaccatttggaggaggacggcggacatgtccaggatgggaatacgcaaaagtggaaatattactgttcctccatcattttgtgaaagcattcagtggttacaccccaactgaccctcatgaaaggatttgtgggtatccagtccctcttgtccctgtcaagggatttccaataaaacttatcgccagatcctga

SEQ ID NO: 11 - protein, 497 aa, Taxus baccata
  source 1..497: note = taxane 10 beta-hydroxylase
MDSFIFLRSIGTKFGQLESSPAILSLTLAPILAIILLLLFRYNHRSSVKLPPGKLGFPLIGETIQLLRTLRSETPQKFFDDRLKKFGPVYMTSLIGHPTVVLCGPAGNKLVLSNEDKLVEMEGPKSFMKLIGEDSIVAKRGEDHRILRTALARFLGAQALQNYLGRMSSEIGHHFNEKWKGKDEVKVLPLVRGLIFSIASTLFFDVNDGHQQKQLHHLLETILVGSLSVPLDFPGTRYRKGLQARLKLDEILSSLIKRRRRDLRSGIASDDQDLLSVLLTFRDEKGNSLTDQGILDNFSAMFHASYDTTVAPMALIFKLLYSNPEYHEKVFQEQLEIIGNKKEGEEISWKDLKSMKYTWQAVQESLRMYPPVFGIFRKAITDIHYDGYTIPKGWRVLCSPYTTHLREEYFPEPEEFRPSRFEDEGRHVTPYTYVPFGGGLRTCPGWEFSKIEILLFVHHFVKNFSSYIPVDPNEKVLSDPLPPLPANGFSIKLFPRS

SEQ ID NO: 12 - RNA, 1494 nt, Taxus baccata
  source 1..1494: mol_type = mRNA; note = taxane 10 beta-hydroxylase
atggatagcttcatttttctgagaagcataggaacaaaatttgggcagctggagtcttcccctgctattctttcccttaccctcgcacctattctcgccattattcttctcttgctcttccgttacaatcaccgatcctctgttaaacttccccctggaaagttaggttttcctctcatcggggagaccatacaattattgcggacactccgatcagaaacacctcaaaagttttttgatgatagattgaagaaattcggtcctgtttacatgacttccctaattgggcatcccacagttgtactctgcgggcctgcgggaaacaaattagttctttcgaacgaggacaagctggtagagatggaagggcccaagtctttcatgaaactgattggggaagattccattgttgctaaaagaggcgaggatcatcgcatcttacgcactgcacttgctcggtttttgggcgctcaagctttacaaaattatctgggtagaatgagttcagaaataggacaccatttcaatgaaaaatggaagggtaaagatgaagtgaaggtgcttcctttggtaagagggcttatcttctccattgcaagcaccctgtttttcgatgtaaatgatggacaccaacagaagcaacttcatcatcttctggaaactattcttgtgggaagtttgtcagtcccgctggactttccaggaactcgttatcgtaaagggcttcaggcgcggctgaagcttgatgaaattctctcctctctaataaaacgcagaagaagagatctgcgttcaggcatagcttctgatgatcaagatctactgtcggtgttgctcaccttcagagatgaaaaagggaactcactgacagaccaggggattctggacaacttttctgctatgtttcatgcttcatatgacaccactgttgcaccaatggccttgatatttaagcttctatactccaatcctgaataccatgaaaaagtatttcaagagcagttggaaataattggcaataaaaaggaaggggaagaaatcagttggaaggatttgaaatctatgaaatatacatggcaagcagttcaagaatcactacgaatgtacccaccagtttttggaatatttcgtaaggctatcactgatattcattatgatgggtatacaattccaaaaggatggagggttttatgttcaccttatactacacatctgagagaagagtacttccctgagcctgaagaattcaggccttcaagatttgaggatgaaggcaggcatgtgactccttacacatatgtaccatttggaggaggcctgcgcacatgtccaggatgggaattttcaaagattgaaatattactgtttgtccatcatttcgttaaaaatttcagcagctacattccagttgatcccaatgaaaaagttttatcagatccactacctcctctccctgccaatggattttccataaaactttttccgagatcctaa

SEQ ID NO: 13 - protein, 485 aa, Taxus baccata
  source 1..485: note = taxane 13 alpha-hydroxylase
MDALKQLEVSPSILFVTLAVMAGIILFFRSKRHSSVKLPPGNLGFPLVGETLQFVRSLGSSTPQQFIEERMSKFGDVFKTSIIGHPTVVLCGPAGNRLVLSNENKLVQMSWPSSMMKLIGEDCLGGKTGEQHRIVRAALTRFLGPQALQNHFAKMSSGIQRHINEKWKGKDEATVLPLVKDLVFSVASRLFFGITEEHLQEQLHNLLEVILVGSFSVPLNIPGFSYHKAIQARATLADIMTHLIEKRRNELRAGTASENQDLLSVLLTFTDERGNSLADKEILDNFSMLLHGSYDSTNSPLTMLIKVLASHPESYEKVAQEQFGILSTKMEGEEIAWKDLKEMKYSWQVVQETLRMYPPIFGTFRKAITDIHYNGYTIPKGWKLLWTTYSTQTKEEYFKDADQFKPSRFEEEGKHVTPYTYLPFGGGMRVCPGWEFAKMETLLFLHHFVKAFSGLKAIDPNEKLSGKPLPPLPVNGLPIKLYSRS

SEQ ID NO: 14 - RNA, 1458 nt, Taxus baccata
  source 1..1458: mol_type = mRNA; note = taxane 13 alpha-hydroxylase
atggatgcccttaagcaattggaagtttccccttccattcttttcgttaccctcgcagtaatggcaggcattatcctcttcttccgctctaaacgccattcctctgtaaaactcccccctggaaatctaggcttccctctggttggggagacactgcagttcgtgaggtcacttggctcgagcactccacagcagtttattgaagagagaatgagcaaatttggggatgtgttcaagacttccataatcgggcatcccacagtagtgctgtgtggacctgccggaaaccggttggttctgtcgaacgagaacaagctggtgcagatgtcatggccgagctccatgatgaaactcatcggcgaagattgtctcggcggcaaaacgggagagcagcatcggatcgtacgcgctgcactaactcggtttttgggtcctcaagcattgcagaatcatttcgctaaaatgagctcgggaatccaacgccacatcaatgaaaaatggaagggaaaggatgaggccactgtacttcctttggtaaaagacctcgtcttctccgtcgcaagccgcttgttttttggtataactgaggagcacctgcaggagcaacttcataacttgttggaagttattcttgtgggatctttttctgttccactcaacattcccggattcagttaccataaagcgattcaggcaagggccaccctcgctgacatcatgacccatttgatagaaaagaggagaaatgagctgcgtgcaggcactgcatctgagaatcaagatttgctctctgttttgctcactttcactgacgaaagggggaattcactggcggacaaggagatcctcgacaacttttctatgttacttcatggatcatatgactccaccaattccccacttaccatgttgattaaagtcttggcctcccatccagaaagctatgaaaaagtggctcaagagcaatttggaatactctccaccaaaatggagggagaagaaattgcttggaaagacctgaaggagatgaaatattcatggcaagttgttcaggaaacattgcgcatgtatcctcccatttttggaacatttcgcaaagccatcactgacattcattacaatggttatacaattccaaaaggatggaaacttttatggacaacttacagtactcaaaccaaggaagagtatttcaaggacgccgatcaattcaagccatcaagatttgaggaggaagggaagcatgtaaccccttacacatacttacctttcggaggaggcatgcgtgtttgtccagggtgggaattcgccaagatggagacattactgtttctccatcattttgttaaagccttctctgggttgaaggcaattgatccaaatgaaaaactttcagggaaaccacttcctcctctccctgtcaatgggcttcccattaaactctattccagatcttaa

SEQ ID NO: 15 - protein, 422 aa, Taxus baccata
  source 1..422: note = Taxane 9 alpha-hydroxylase
MPIQMDTLIQIQSSPVFLSFTLTAFLGVVVLLIFRYKHRSALKLPPGNLGLPFIGETITFASQPPQKFLNERRKKFGPVFKTSLIGHPTVVLCGSSGNRFLLSNEEKLVRMSLPNSYMKLLGQDSLLGKTGEEHRIVRTALGRFLGPQELQNHVAKMSSDIQHHINQKWKGNDEVKVLPLIRNLVFSIATSLFFGINDEHQQERLHLLLETIVMGAVCIPLAFPGSGFRKALQARSELDGILISLMKIRRSDLRSGAASSNQDLLSVLLTFKDERGNPLTDKEILDNFSVLLHGLYDTTISPLTLIFKLMSSNTECYENVVQGMQSLKLFLSSLYVLINRLCNLCLHVLGVYITEQLEILSHKEKGEEIGWKDLKSMKYTWQAIQETLRMFPPVYGNFRKALTDIHYDGYTIPKGWRVSFSH

SEQ ID NO: 16 - RNA, 1645 nt, Taxus baccata
  source 1..1645: mol_type = mRNA
atgcccatccaaatggataccttaattcagatccagtcttcccctgttttcctttcctttactctcacagcgtttctgggcgttgttgtgcttttgatattccgttataaacaccgatccgctctcaaacttccacctggaaatttaggcttgcccttcattggggagacaataacatttgcatctcaacctcctcagaagtttttaaacgagaggaggaagaaatttggtcctgttttcaagacgtcgctaattgggcatcccacagttgttctctgcggctcctcgggaaaccgttttctcctctccaacgaggaaaagctggtgcggatgtctttgcccaactcatacatgaaactcctggggcaggattcccttctggggaaaacgggagaggaacatcggattgtgcgtaccgcactaggacgttttttgggcccccaagagttgcagaatcatgtggccaagatgagttcagacattcagcatcacatcaaccaaaaatggaaggggaatgatgaagtgaaggtgcttcctctgataaggaaccttgtcttctccattgcaaccagcttgtttttcggtataaacgatgagcaccaacaggagcgacttcatcttcttttggaaactattgtaatgggagctgtgtgtattccgctcgcctttccaggatctggttttcgtaaagcgcttcaggcacggtcggagctcgatggaattctcatttctttaatgaaaatcagaagaagcgatctgcgttcaggcgcagcttcaagcaaccaagatctactgtcggtgttgctcaccttcaaagatgaaagagggaatccattgacagacaaggagatcctcgacaacttctctgttctacttcatggcttatatgacaccacaatttcaccactcaccttgatttttaagctcatgtcctccaatactgaatgctacgagaatgtagtccaaggtatgcaaagcctcaaactttttctttcatctctatatgtgcttattaataggctatgcaatttatgtctacatgtgttgggtgtatatattacagagcaattagaaatactttcccataaagagaagggagaggagatcggttggaaggatctgaaatctatgaaatatacttggcaagccattcaggaaaccttgagaatgttccctccggtttacggaaattttcgcaaggctttgactgatattcattacgatggctatacaatcccaaaagggtggagggtaagcttttctcattaaatcaattcaataattcgatgtttttttttcttggattaatattagttctgctatatgttgtgaacaggttttattttcgccttttaccacgcacagcaatgaagaatattttaatgagccagatgaattcagaccttcaagattcgaggggcaaggaaagaatgtggcttcttacacattcataccgttcggaggaggcctgcgcatatgtccaggatgggaatttgcaaagacagagatgttactgtttatacattattttgttaaaactttcagcagctacgtcccagttgaccccaacgaaaagatttcagcagatccgctcgcttctttccctgttaatggattttccgtaaaactttttccaaggtcctaa

SEQ ID NO: 17 - protein, 348 aa, Taxus baccata
  source 1..348: note = taxane 1 beta-hydroxylase
MDSFNFLRGIGADFGGFIQFQSSPAVLSLSLITTILGVLLLWFFLHKNGSSVTLPPGNLGFPFIGETIPFLRALRSETPQTFFDERVKKFGVVFKTRIVGHPTVVLCGPEGNRFLLSNEDKLVQASLPNSSQKLIGKYSILSKRGEEHRILRAALARFLRPQALQGYVAKMSSEIQHHIKQKWKGNDEVKVLPLIRTLIFNIASSLFFGINDEHQQEQLHHFLEAIVLGSLSVPLDFPGTRFRKALDARSKLDEILSSLMESRRRDLRLGTASENQDLLSVLLTFKDERGNPLTDKEILDNFSFMLHASYDTTVSPTVLMLKLLFSSPDYYEKLVQGMPNPYYFLSVL

SEQ ID NO: 18 - RNA, 1680 nt, Taxus baccata
  source 1..1680: mol_type = mRNA; note = taxane 1 beta-hydroxylase
atggatagcttcaatttcttgagaggcattggagcagattttgggggattcattcagttccagtcttcccctgctgttctttccctttccctgatcacaactattcttggcgttctacttctctggttcttccttcataaaaacggttcctctgttactctcccccctggaaatttaggcttccctttcattggggagaccataccattcttgagggcacttcgatcagaaacacctcagacgttttttgatgagagagtgaagaaattcggtgttgtattcaagactcggatagttgggcatcccacagttgtactctgcgggcctgagggaaaccgctttcttctctccaacgaggacaaactggtgcaggcgtcattgcccaactcttcccagaaactaattgggaaatattccattctgtccaaaagaggggaggagcatcgcatattacgtgctgcacttgcccgctttttgcgaccccaagctttgcagggttatgttgctaaaatgagttcagaaatccaacatcatatcaagcaaaaatggaagggaaatgatgaagtgaaggtgcttcctctgataagaaccctgatcttcaacattgcaagcagcctgtttttcggcataaatgatgaacaccaacaggaacagcttcatcattttttggaagccattgttctgggaagtctgtctgttccgctcgactttccaggaactcgttttcgtaaagctcttgatgcgcggtctaagctggatgagattctttcttctttaatggagagcagaagaagggatctgcgtttgggcacggcttctgagaatcaagatcttctttctgtgttgctcaccttcaaagatgaaagagggaatccactcacagacaaggaaatcctcgacaatttttcatttatgcttcatgcctcgtatgataccactgtttcaccaacggttttgatgcttaagcttctcttctctagtcctgattactatgaaaaactagttcaaggtatgccaaacccatattattttctctctgttctataataatgtgcgttttaatttataagtgacatggggtatatgtattgtaataacagaacaattgggaatagttggcaataaaaaggagggagaagaaatcagctggaacgatctgaaagctatgaaatatacatggcaagttgtgcaggaaactatgaggatgctccctccagtttttggatcgtatcgcaaggctataaccgatatccattatgatgggtatacaattccaaaaggatggaatgtaagctgtttccattaaatcaattcaattcatattttaggaaagacaaaaaaaatctaatccgactctgatgattttgtgagcagatattctggtcaccttatactacacacgggaaagaagaatacttcaatgaagcggagaagttcatgccttcaagattcgaggaaggcaaatatgttgctccttacactttcttgccattcggagcaggtctgcgcgtatgtccaggatgggaatttgcaaagaccgagatattactgttcgtccatcattttgttacaactttcagcagctacatcccaattgaccccaaagagaaaatttcaggggatccatttcctcctctgcctaccaatggattttccgtgaaactttttaccagatcttaa

SEQ ID NO: 19 - protein, 439 aa, Taxus baccata
  source 1..439: note = taxadiene-5 alpha-ol-O-acetyl transferase
MEKTDLHVNLIEKVMVGPSPPLPKTTLQLSSIDNLPGVRGSIFNALLIYNASPSPTMISADPAKPIREALAKILVYYPPFAGRLRETENGDLEVECTGEGAMFLEAMADNELSVLGDFDDSNPSFQQLLFSLPLDTNFKDLSLLVVQVTRFTCGGFVVGVSFHHGVCDGRGAAQFLKGLAEMARGEVKLSLEPIWNRELVKLDDPKYLQFFHFEFLRAPSIVEKIVQTYFIIDFETINYIKQSVMEECKEFCSSFEVASAMTWIARTRAFQIPESEYVKILFGMDMRNSFNPPLPSGYYGNSIGTACAVDNVQDLLSGSLLRAIMIIKKSKVSLNDNFKSRAVVKPSELDVNMNHENVVAFADWSRLGFDEVDFGWGNAVSVSPVQQQSALAMQNYFLFLKPSKNKPDGIKILMFLPLSKMKSFKIEMEAMMKKYVAKV

SEQ ID NO: 20 - RNA, 1320 nt, Taxus baccata
  source 1..1320: mol_type = mRNA; note = taxadiene-5 alpha-ol-O-acetyl transferase
atggagaagacagatttacacgtaaatctgattgagaaagtgatggttgggccatccccgcctctgcccaaaaccaccctgcaactctcctccatagacaacctgccaggggtaagaggaagcattttcaatgccttgttaatttacaatgcctctccctctcccaccatgatctctgcagatcctgcaaaaccaattagagaagctctcgccaagatcctggtttattatcccccttttgctgggcgcctcagagagacagaaaatggggatctggaagtggaatgcacaggggagggtgctatgtttttggaagccatggcagacaatgagctgtctgtgttgggagattttgatgacagcaatccatcatttcagcagctacttttttcgcttccactcgataccaatttcaaagacctctctcttctggttgttcaggtaactcgttttacatgtggaggctttgttgttggagtgagtttccaccatggtgtatgtgatggtcgaggagcggcccaatttcttaaaggtttggcagagatggcacggggagaggttaagctctcattggaaccaatatggaatagggaactagtgaagcttgatgaccctaaataccttcaattttttcactttgaattcctacgagcgccttcaattgttgagaaaattgttcaaacatattttattatagattttgagaccataaattatatcaaacaatctgttatggaagaatgtaaagaattttgctcttcattcgaagttgcatcagcaatgacttggatagcaaggacaagagcttttcaaattccagaaagtgagtacgtgaaaattctcttcggaatggacatgaggaactcatttaatccccctcttccaagcggatactatggtaactccattggtaccgcatgtgcagtggataatgttcaagacctcttaagtggatctcttttgcgtgctataatgattataaagaaatcaaaggtctctttaaatgataatttcaagtcaagagctgtggtgaagccatctgaattggatgtgaatatgaatcatgaaaacgtagttgcatttgctgattggagccgattgggatttgatgaagtggattttggttgggggaatgcggtgagtgtaagccctgtgcaacaacagtctgcgttagcaatgcaaaattattttcttttcctaaaaccttccaagaacaagcccgatggaatcaaaatattaatgtttctgcccctatcaaaaatgaagtcattcaaaattgaaatggaagccatgatgaaaaaatatgtggctaaagtatga

SEQ ID NO: 21 - protein, 440 aa, Taxus baccata
  source 1..440: note = taxane-2 alpha-O-benzoyltransferase
MGRFNVDMIERVIVAPCLQSPKNILHLSPIDNKTRGLTNILSVYNASQRVSVSADPAKTIREALSKVLVYYPPFAGRLRNTENGDLEVECTGEGAVFVEAMADNDLSVLQDFNEYDPSFQQLVFNLREDVNIEDLHLLTVQVTRFTCGGFVVGTRFHHSVSDGKGIGQLLKGMGEMARGEFKPSLEPIWNREMVKPEDIMYLQFDHFDFIHPPLNLEKSIQASMVISFERINYIKRCMMEECKEFFSAFEVVVALIWLARTKSFRIPPNEYVKIIFPIDMRNSFDSPLPKGYYGNAIGNACAMDNVKDLLNGSLLYALMLIKKSKFALNENFKSRILTKPSTLDANMKHENVVGCGDWRNLGFYEADFGWGNAVNVSPMQQQREHELAMQNYFLFLRSAKNMIDGIKILMFMPASMVKPFKIEMEVTINKYVAKICNSKL

SEQ ID NO: 22 - RNA, 1367 nt, Taxus baccata
  source 1..1367: mol_type = mRNA; note = taxane-2 alpha-O-benzoyltransferase
atgggcaggttcaatgtagatatgattgagcgagtgatcgtggcgccatgccttcaatcgcccaaaaatatcctgcacctctcccccattgacaacaaaactagaggactaaccaacatattatcagtctacaatgcctcccagagagtttctgtttctgcagatcctgcaaaaacaattcgagaggctctctccaaggtgctggtttattatcccccttttgctggaaggctgagaaacacagaaaatggggatcttgaagtggagtgcacaggggagggtgccgtctttgtggaagccatggcggacaacgacctttcagtattacaagatttcaatgagtacgatccatcatttcagcagctagtttttaatcttcgagaggatgtcaatattgaggacctccatcttctaactgttcaggtaactcgttttacatgtggaggatttgttgtgggcacaagattccaccatagtgtatctgatggaaaaggaatcggccagttacttaaaggcatgggagagatggcaaggggggagtttaagccctcgttagaaccaatatggaatagagaaatggtgaagcctgaagacattatgtacctccagtttgatcactttgatttcatacacccacctcttaatcttgagaagtctattcaagcatctatggtaataagctttgagagaataaattatatcaaacgatgcatgatggaagaatgcaaagaatttttttctgcatttgaagttgtagtagcattgatttggctggcaaggacaaagtcttttcgaattccacccaatgagtatgtgaaaattatctttccaatcgacatgaggaattcatttgactcccctcttccaaagggatactatggtaatgctattggtaatgcatgtgcaatggataatgtcaaagacctcttaaatggatctcttttatatgctctaatgcttataaagaaatcaaagtttgctttaaatgagaatttcaaatcaagaatcttgacaaaaccatctacattagatgcgaatatgaagcatgaaaatgtagtcggatgtggcgattggaggaatttgggattttatgaagcagattttggatggggaaatgcagtgaatgtaagccccatgcagcaacaaagagagcatgaattagctatgcaaaattattttctttttctccgatcagctaagaacatgattgatggaatcaagatactaatgttcatgcctgcatcaatggtgaaaccattcaaaattgaaatggaagtcacaataaacaaatatgtggctaaaatatgtaactctaagttataaagtatgtatgactgcaaaatagtaaaatattgcatggtggatgc

SEQ ID NO: 23 - protein, 393 aa, Taxus baccata
  source 1..393: note = geranylgeranyl diphosphate synthase
MAYTAMAAGTQSLQLRTVASYQECNSMRSCFKLTPFKSFHGVNFNVPSLGAANCEIMGHLKLGSLPYKQCSVSSKSTKTMAQLVDLAETEKAEGKDIEFDFNEYMKSKAVAVDAALDKAIPLEYPEKIHESMRYSLLAGGKRVRPALCIAACELVGGSQDLAMPTACAMEMIHTMSLIHDDLPCMDNDDFRRGKPTNHKVFGEDTAVLAGDALLSFAFEHIAVATSKTVPSDRTLRVISELGKTIGSQGLVGGQVVDITSEGDANVDLKTLEWIHIHKTAVLLECSVVSGGILGGATEDEIARIRRYARCVGLLFQVVDDILDVTKSSEELGKTAGKDLLTDKATYPKLMGLEKAKEFAAELATRAKEELSSFDQIKAAPLLGLADYIAFRQN

SEQ ID NO: 24 - RNA, 1182 nt, Taxus baccata
  source 1..1182: mol_type = mRNA; note = geranylgeranyl diphosphate synthase
atggcttacacggcaatggcagcagggacccaaagcttgcaactccgcactgttgcttcctatcaagaatgcaatagtatgaggagttgttttaaattgacaccttttaaaagttttcatggagtgaatttcaatgttccctcactgggtgctgctaattgtgagattatgggtcacctgaaacttgggtcattgccatataaacaatgttcggtgtcatctaaatccacaaaaacaatggcccagttggttgatttggctgaaacagagaaggcggagggaaaggatattgaatttgatttcaacgagtatatgaagtccaaggctgtggcagtggatgcggcactggataaggcaatcccacttgaatatcctgaaaaaatacatgaatcaatgaggtattcacttctagcaggaggtaagcgcgtcaggcctgctctgtgcattgcagcatgtgagcttgtaggagggagtcaggaccttgccatgccaactgcctgtgcaatggagatgattcataccatgtctctgattcatgatgacttgccgtgcatggataatgatgatttcagaagagggaagccaacaaatcacaaggtctttggagaggacactgctgttcttgcaggggacgccctgctttcatttgcatttgagcatattgctgtggctacaagcaagactgtgcctagtgataggactttaagggtgatatctgaattgggtaagacaataggctctcaagggcttgtaggggggcaggtggttgatattacatccgagggggatgctaatgtggacctgaaaaccctggaatggattcatatacacaagactgctgtgctcttggaatgttcagttgtgagtggagggatccttggtggtgctacagaggacgagattgcgagaattcggcggtacgcccggtgtgtggggcttctgtttcaggttgtggatgacatacttgatgtcactaaatcttctgaagaattgggaaagactgcaggaaaggatttgcttactgataaggctacttatcccaagttgatgggcctggagaaagcaaaagaatttgccgctgaattggcgacgagagccaaggaagagctgtcatcctttgatcagataaaggctgcacctttgttgggtcttgcagattacattgcattcaggcaaaactga

SEQ ID NO: 25 - protein, 318 aa, Taxus baccata
  source 1..318: note = taxane 9 alpha-dioxygenase1
MDSSLEKEVDLPFIDLSQFSFDSEGIKNLQNHPGVATVRESCQEWGFFRIMNTGIPNDVFQKVESVSHELFAMPQEMKDRAITSSPHDTYINHPYRESFWFPTPPHSDSVLAFCNKLWPEKDNLKLCETIGAYILSMEDLKRKISSIIIASLGLDKVETFYHSDFEKGTSVFRIHHYYSDGKFAAGEQALFAHTDPHCFTILYQDNGAGLQIQSKEGNWVHVKHIPNSLIINVADSLKAWSNGRYRSVNHRVVYKDWTNRISLGWFMMFPDKEIRVPAELIDDQHPQCYRPFTYLQFRDAFMKDRIDIDGYAGIIPTY

SEQ ID NO: 26 - RNA, 957 nt, Taxus baccata
  source 1..957: mol_type = mRNA; note = taxane 9 alpha-dioxygenase1
atggattcctcgctggagaaagaagttgatcttccatttatcgacctctcacagttttctttcgactccgagggaatcaaaaaccttcaaaaccatccgggggtagccacagtgagggaatcctgccaagaatggggattcttccgcattatgaacactggaattccaaatgatgttttccagaaggtggagagtgttagccacgagctgtttgccatgccacaggagatgaaggacagagccatcacatccagcccgcatgacacctacattaatcacccttacagggaaagcttctggttcccaactccgcctcattccgattccgtcctcgccttctgtaacaagctatggccggaaaaggataaccttaagttgtgcgagacaattggagcatatatacttagcatggaggacctgaaacgcaagataagtagtatcattatagccagtttggggttagacaaggtggaaactttttaccattctgatttcgaaaaaggcacatctgttttccgtatacaccactattactccgatggaaaattcgcagctggcgaacaagctctgtttgcgcacaccgatccccattgttttaccatcctttaccaagacaatggcgcggggctccagattcaatccaaggaaggcaactgggttcacgtcaaacatatccccaattccttgattatcaacgtagctgactccctaaaggcatggagcaatggcaggtaccgcagcgtaaatcatcgcgttgtttacaaagattggacgaatcgcatatctttagggtggtttatgatgtttccagacaaggaaatacgggttccggctgaattaatagacgaccaacatccacaatgttaccgcccttttacttacctccagttccgagatgcttttatgaaagatcgcatagatattgatggctatgcaggcataattcctacttattga

SEQ ID NO: 27 - protein, 440 aa, Taxus baccata
  source 1..440: note = 10-deacetyl baccatin III-10-O-acetyltransferase
MAGSTEFVVRSLERVMVAPSQPSPKAFLQLSTLDNLPGVRENIFNTLLVYNASDRVSVDPAKVIRQALSKVLVYYSPFAGRLRKKENGDLEVECTGEGALFVEAMADTDLSVLGDLDDYSPSLEQLLFCLPPDTDIEDIHPLVVQVTRFTCGGFVVGVSFCHGICDGLGAGQFLIAMGEMARGEIKPSSEPIWKRELLKPEDPLYRFQYYHFQLICPPSTFGKIVQGSLVITSETINCIKQCLREESKEFCSAFEVVSALAWIARTRALQIPHSENVKLIFAMDMRKLFNPPLSKGYYGNFVGTVCAMDNVKDLLSGSLLRVVRIIKKAKVSLNEHFTSTIVTPRSGSDESINYENIVGFGDRRRLGFDEVDFGWGHADNVSLVQHGLKDVSVVQSYFLFIRPPKNNPDGIKILSFMPPSIVKSFKFEMETMTNKYVTKP

SEQ ID NO: 28 - RNA, 1488 nt, Taxus baccata
  source 1..1488: mol_type = mRNA; note = 10-deacetyl baccatin III-10-O-acetyltransferase
gcaccagctgagcttgatctgagatggcaggctcaacagaatttgtggtaagaagcttagagagagtgatggtggctccaagccagccatcgcccaaagctttcctgcagctctccacccttgacaatctaccaggggtgagagaaaacatttttaacaccttgttagtctacaatgcctcagacagagtttccgtagatcctgcaaaagtaattcggcaggctctctccaaggtgttggtgtactattccccttttgcagggcgtctcaggaaaaaagaaaatggagatcttgaagtggagtgcacaggggagggtgctctgtttgtggaagccatggctgacactgacctctcagtcttaggagatttggatgactacagtccttcacttgagcaactacttttttgtcttccgcctgatacagatattgaggacatccatcctctggtggttcaggtaactcgttttacatgtggaggttttgttgtaggggtgagtttctgccatggtatatgtgatggactaggagcaggccagtttcttatagccatgggagagatggcaaggggagagattaagccctcctcggagccaatatggaagagagaattgctgaagccggaagaccctttataccggttccagtattatcactttcaattgatttgcccgccttcaacattcgggaaaatagttcaaggatctcttgttataacctctgagacaataaattgtatcaaacaatgccttagggaagaaagtaaagaattttgctctgcgttcgaagttgtatctgcattggcttggatagcaaggacaagggctcttcaaattccacatagtgagaatgtgaagcttatttttgcaatggacatgagaaaattatttaatccaccactttcgaagggatactacggtaattttgttggtaccgtatgtgcaatggataatgtcaaggacctattaagtggatctcttttgcgtgttgtaaggattataaagaaagcaaaggtctctttaaatgagcatttcacgtcaacaatcgtgacaccccgttctggatcagatgagagtatcaattatgaaaacatagttggatttggtgatcgaaggcgattgggatttgatgaagtagactttgggtgggggcatgcagataatgtaagtctcgtgcaacatggattgaaggatgtttcagtcgtgcaaagttattttcttttcatacgacctcccaagaataaccccgatggaatcaagatcctatcgttcatgcccccgtcaatagtgaaatccttcaaatttgaaatggaaaccatgacaaacaaatatgtaactaagccttgaaattgtagtaacttaagccttgcattttcagaataagttttggcactgggttgtggttgaagtaatgtacttttgaattttgatttaaagttctattcaaagttataaaatgtattatgtgaaaatatgttgcaattatggt

SEQ ID NO: 29 - protein, 445 aa, Taxus baccata
  source 1..445: note = baccatin III-3-amino, 13-phenylpropanoyltransferase
MKKTGSFAEFHVNMIERVMVRPCLPSPKTILPLSAIDNMARAFSNVLLVYAANMDRVSADPAKVIREALSKVLVYYYPFAGRLRNKENGELEVECTGQGVLFLEAMADSDLSVLTDLDNYNPSFQQLIFSLPQDTDIEDLHLLIVQVTRFTCGGFVVGANVYGSACDAKGFGQFLQSMAEMARGEVKPSIEPIWNRELVKLEHCMPFRMSHLQIIHAPVIEEKFVQTSLVINFEIINHIRRRIMEERKESLSSFEIVAALVWLAKIKAFQIPHSENVKLLFAMDLRRSFNPPLPHGYYGNAFGIACAMDNVHDLLSGSLLRTIMIIKKSKFSLHKELNSKTVMSSSVVDVNTKFEDVVSISDWRHSIYYEVDFGWGDAMNVSTMLQQQEHEKSLPTYFSFLQSTKNMPDGIKMLMFMPPSKLKKFKIEIEAMIKKYVTKVCPSKL

SEQ ID NO: 30 - RNA, 1338 nt, Taxus baccata
  source 1..1338: mol_type = mRNA; note = baccatin III-3-amino, 13-phenylpropanoyltransferase
atgaagaagacaggttcgtttgcagagttccatgtgaatatgattgagcgagtcatggtgagaccgtgcctgccttcgcccaaaacaatcctccctctctccgccattgacaacatggcaagagctttttctaacgtattgctggtctacgctgccaacatggacagagtctctgcagatcctgcaaaagtgattcgagaggctctctccaaggtgctggtttattattacccttttgctgggcggctcagaaataaagaaaatggggaacttgaagtggagtgcacagggcagggtgttctgtttctggaagccatggctgacagcgacctttcagtcttaacagatctggataactacaatccatcgtttcagcagttgattttttctctaccacaggatacagatattgaggacctccatctcttgattgttcaggtaactcgttttacatgtgggggttttgttgtgggagcgaatgtgtatggtagtgcatgcgatgcaaaaggatttggccagtttcttcaaagtatggcagagatggcgagaggagaggttaagccctcgattgaaccgatatggaatagagaactggtgaagctagaacattgtatgcccttccggatgagtcatcttcaaattatacatgcacctgtaattgaggagaaatttgttcaaacatctcttgttataaactttgagataataaatcatatcagacgacgcatcatggaagaacgcaaagaaagtttatcttcatttgaaattgtagcagcattggtttggctagcaaagataaaggcttttcaaattccacatagtgagaatgtgaagcttctttttgcaatggacttgaggagatcatttaatccccctcttccacatggatactatggcaatgcctttggtattgcatgtgcaatggataatgtccatgaccttctaagtggatctcttttgcgcactataatgatcataaagaaatcaaagttctctttacacaaagaactcaactcaaaaaccgtgatgagctcatctgtagtagatgtcaatacgaagtttgaagatgtagtttcaattagtgattggaggcattctatatattatgaagtggactttgggtggggagatgcaatgaacgtgagcactatgctacaacaacaggagcacgagaaatctctgccaacttatttttctttcctacaatctactaagaacatgccagatggaatcaagatgctaatgtttatgcctccatcaaaactgaaaaaattcaaaattgaaatagaagctatgataaaaaaatatgtgactaaagtgtgtccgtcaaagttatga

SEQ ID NO: 31 - protein, 698 aa, Taxus baccata
  source 1..698: note = phenylalanineaminomutase
MGFAVESRSHVKDILGLINTFNEVKKITVDGTTPITVAHVAALARRHDVKVALEAEQCRARVETCSSWVQRKAEDGADIYGVTTGFGACSSRRTNQLSELQESLIRCLLAGVFTKGCASSVDELPATATRSAMLLRLNSFTYGCSGIRWEVMEALEKLLNSNVSPKVPLRGSVSASGDLIPLAYIAGLLIGKPSVVARIGDDVEVPAPEALSRVGLRPFKLQAKEGLALVNGTSFATALASTVMYDANVLLLLVETLCGMFCEVIFGREEFAHPLIHKVKPHPGQIESAELLEWLLRSSPFQDLSREYYSIDKLKKPKQDRYALRSSPQWLAPLVQTIRDATTTVETEVNSANDNPIIDHANDRALHGANFQGSAVGFYMDYVRIAVAGLGKLLFAQFTELMIEYYSNGLPGNLSLGPDLSVDYGLKGLDIAMAAYSSELQYLANPVTTHVHSAEQHNQDINSLALISARKTEEALDILKLMIASHLTAMCQAVDLRQLEEALVKVVENVVSTLADECGLPNDTKARLLYVAKAVPVYTYLESPCDPTLPLLLGLEQSCFGSILALHKKDGIETDTLVDRLAEFEKRLSDRLENEMTAVRVLYEKKGHKTADNNDALVRIQGSRFLPFYRFVREELDTGVMSARREQTPQEDVQKVFDAIADGRITVPLLHCLQGFLGQPNGCANGVESFQSVWNKSA

SEQ ID NO: 32 - RNA, 2097 nt, Taxus baccata
  source 1..2097: mol_type = mRNA; note = phenylalanineaminomutase
atggggtttgccgtggaatcgcgttctcacgtaaaggatatattggggctgatcaacacgttcaacgaggtgaagaaaattacagtagacggtacgacccccatcacggtggcccatgtcgcggcgctggcccggaggcatgacgtgaaggttgcgttggaggcggagcaatgcagagcccgtgtggaaacctgctcttcgtgggtgcagcgcaaggcggaagacggcgccgacatatacggcgtcaccacgggctttggcgcgtgctcgagccgtaggaccaaccagctgagcgagctgcaggagtcgcttatacgctgcctgctcgcgggggtgtttactaaaggatgcgcttcctccgtcgacgagctccctgcgaccgccacccgcagcgccatgctgctccgccttaatagttttacctatggatgttccggcatccggtgggaggtcatggaagcgctggaaaagcttctcaacagcaatgtctctcctaaagtgcctctccgaggatctgtgagcgcttcgggagacctcatcccgctcgcctacattgcagggctcctgattgggaagcctagcgtagtcgctcgcataggcgacgatgtcgaggtccctgcgcccgaagcgttgagcagggtggggctgcggccattcaagctccaggccaaagaagggctggcgctcgtcaacggcacctccttcgccaccgcgctcgcctccaccgtcatgtacgacgccaatgttctgttgctgctcgtcgaaacgctttgcggaatgttctgcgaggtgatctttggaagggaggagttcgcgcatccgctgatccataaagtgaagccgcacccaggccagatcgaatcggcggagctgctcgagtggctgctgcggtcgagcccgtttcaggacctgtcgagggagtattacagtattgataagctgaagaaaccgaaacaggatcgctatgctctgaggtcgagcccgcagtggttggctcctctggtgcagacaatcagagacgccaccactacagtggagacggaggtcaattccgccaatgataaccccatcattgaccacgccaatgacagggctctccatggtgcgaatttccagggcagcgccgtcggcttctacatggactacgtgcgcatcgcagtcgccgggctggggaaactcttgttcgctcagttcacggagctgatgatcgaatattacagcaacggcctaccggggaacctctccctggggccggacctgagcgtggactacggcctcaaggggctcgacatcgccatggccgcctacagctccgagcttcagtacctggcgaatcccgtgaccacacacgtgcacagcgcggaacagcacaaccaggacatcaactctctggcgctcatctccgcccgcaagacggaggaagcgttggatatcttaaagctcatgatcgcctcgcatttaacagcaatgtgccaggcggtggaccttcggcagctcgaagaagccctagtaaaagtcgtggagaatgtcgtttccacccttgcagacgaatgcggcctccctaacgacacaaaggcgaggcttttatatgtagccaaagcggtgcctgtttacacatacctggaatccccctgcgaccctacgcttcccctcttgttaggcctggaacagtcctgtttcggttccattctggctctccacaaaaaagacggcattgagacggacaccttggtcgatcggctcgccgagttcgagaagcggctgtccgaccgcctggaaaacgagatgacggcagtgagggttttgtacgaaaagaaagggcataaaactgcagacaacaacgacgccctcgtgagaatccagggttccagattccttcctttttacagatttgttcgggaagagctcgacacaggtgtgatgagtgcgagaagagagcagacgccgcaagaggacgtgcagaaagtgttcgatgcaattgccgacggcagaattacggtgcctctgctgcactgcctgcaagggtttctcggccaaccaaatgggtgcgccaacggcgtcgagtcgttccaaagtgtttggaacaaatctgcgtga

SEQ ID NO: 33 - protein, 555 aa, Taxus baccata
  source 1..555: note = phenylalanine-CoA ligase
MAAPGLEVDPRSGSCNTNATFYSKRKPLNVPQEEYLDLPTFVSRHPHTGKIALIDSSTGNKITFPQLWHNVKSLAAGLSQSGVKMGDVVLLLSPNSIHFPIICMAIMSIGAVVTTTNPLNTAAEIAKQAADSHAVLAFVTPELANKLAATNLSLVFIPTPTTRSLSDLVAGDTPKSPAIRSLLDLMAADPAKAPTVKISQDDTATLLYSSGTTGLSKGVISTHRNLISMVCVLLSRFNLSGTSNNSFLCTVPMFHIYGLAAFACGLLASGSTIVVLSKFELGEMLGAIEKYRVTYLPLVPPILLALTKTEICRKYDLRSLHTVLCGGAPLSKESTEEFISRFPTIKLMQGYGLTETTAIGASTDTQEESRHYGTAGMLSPNTDAKIVDPDSGLALPPNHRGELWLRGPTIMKGYFSNPEATSSAMDRSGWLRTGDLCYIDTEGYVFVVDRLKELIKYKGYQVAPAELEALLLSHPEIADVAVIPFPDKEAGQVPMAYIVRKQGSTLSEASVIGFVAKQVAPYKKVRRVAFVSGIPKNAPGKILRKDLIKLSTSRL

SEQ ID NO: 34 - RNA, 1668 nt, Taxus baccata
  source 1..1668: mol_type = mRNA; note = phenylalanine-CoA ligase
atggcagcaccaggtctcgaggtcgatccccgcagcgggtcctgcaacacaaatgccactttctacagcaagcgaaagcccttaaacgtcccccaagaagaatatctggacctcccaaccttcgtctcacgacaccctcacacagggaaaatagccctcatagactcctccacaggcaacaaaatcacctttccccagctatggcacaatgtcaaatccttggcagcaggtttatcccaatccggtgtcaaaatgggcgacgtggtcctcctcctctccccgaattcaatccatttccccatcatttgcatggcgatcatgtccatcggcgccgtagtcaccacgaccaatcctctcaataccgctgcagaaattgcaaagcaagccgctgactcgcatgcagttttggcgtttgtaacgccagaactagcaaacaagttagcagcaaccaacttaagcttggttttcataccaaccccgaccacaaggtctttgtcagatcttgtggcgggggatacccccaagtcccccgccataaggtctttgttagaccttatggcagcagaccccgccaaggcccccactgtcaaaatcagccaagatgacactgccaccttactgtactcttctggcaccactggtctcagcaaaggagtcatctccacccatagaaacctcatatccatggtctgtgttttgctgagcaggttcaatttgtctggcacctctaacaattcttttctgtgcactgtgccaatgtttcatatttatggccttgcagcttttgcatgtgggctgcttgcctctgggtctactattgttgtgctgtctaagtttgaattgggggagatgcttggggctattgagaagtatagggtgacttatttgccacttgtgccaccgattttgctggcactcacaaaaacagagatttgtaggaagtatgatctgaggtctctgcatactgtgctttgtggcggggctcccctcagtaaggagtccactgaagagtttatttctaggtttcccacaatcaaattaatgcagggttatgggctgacagaaacaactgcaataggagcatccacagacacccaagaggagagcagacactatggaacagctggcatgctgtccccaaatactgatgcaaagattgtggatcctgattctggtcttgctctccctccaaatcatagaggagagttgtggctacgtggcccaacaattatgaaaggttacttcagcaatccagaagctactagttcagctatggaccgaagtggctggctccgtacaggtgatctctgctacattgatactgaaggctatgtctttgtagtagacagactgaaagagttgataaaatacaaaggctatcaggttgctccggcagaattagaagcacttctgctttctcatcctgagatcgctgatgtcgcagtgataccgtttccagacaaagaagcaggccaggttccaatggcgtacatcgtaaggaaacagggcagcacactgtctgaagctagtgtcattggttttgttgccaaacaggtggcaccatacaagaaagttcgcagggtggcttttgtgagtggaattccaaaaaatgccccgggaaagatattaagaaaggatttgatcaaactatccacatcaagactttga

SEQ ID NO: 35 - protein, 515 aa, Taxus baccata
  source 1..515: note = taxane 2 alpha-hydroxylase
MASFLNQSFLSVSSLVSSSPLQMAAIIFVTVLVIARIGRKGSKLPPGPLSLPIFGNWLQVGNDLNHRNLMMLAKKYGDVFMLRLGCRNLVVVSSPELAKQVLHTQGIEFGSRKNNLVFDIFTGNGQDMVFTVYGEHWRKMRRIMTLPFFTQKVVHYYREGWEDEIQKAVEDVRANETAFRSGIVIRKRLQLMLYNVMYRMMFDRRFESQEDPLFVQAISFNAQRSQLAQSFEYNYGDFIPILRPFLRGYLNKCKDLQSRRLAFFNDIFIQERRKILEKGEQMTTKCAIDHILEAEKKGEINEKNVVYIVENINVAAIETTLWSMEWALAELVNHPEVQRKVRSEVESIVGRGAAVKEADIEKLPYLQAVVKETLRLHTPIPLLVPHMNLDDASLGGFSIPRESKVVVNAWWLANNPEWWDDPSEFRPERFMEEERETEAAVGGKVDFRFLPFGMGRRSCPGIILALPVLGLVIGRLLQNFELIPPPGREKIDLSEKGGQFSLHIATHSTIRFRLI

SEQ ID NO: 36 - RNA, 1595 nt, Taxus baccata
  source 1..1595: mol_type = mRNA; note = taxane 2 alpha-hydroxylase
aagtgtgttgttttcaccttcaatttgaacaatggcgtcttttcttaaccagagttttctctctgtttcttcacttgtttcttcttctccattacaaatggctgcaatcatatttgtgacggtgttagtcatagccagaattggtaggaaaggctcgaaactgcctcccggcccgctgtctttgcccatatttggcaactggctgcaagtcggcaacgatctaaaccacagaaatctgatgatgttggcgaagaagtatggagacgttttcatgctgagattggggtgcagaaatttagtggtggtgtcgtctccggagctcgccaaacaagttctgcatacgcagggcatcgagttcggttcgagaaagaacaatctggttttcgacattttcacggggaacgggcaagacatggtgttcactgtgtatggagagcactggcgaaagatgcgaagaatcatgacgcttcccttctttactcagaaagttgtccactattacagagaaggttgggaggatgagatccagaaagccgtcgaagatgttcgggcgaacgaaacggcgttccgcagcgggattgtgataagaaaacggcttcagctcatgctttataatgttatgtatcggatgatgtttgatcgcaggttcgagtctcaggaggatccgctgtttgtccaggcgatttcttttaatgcgcagagaagtcaactcgcgcaaagcttcgagtacaattatggggatttcattcccatcttgaggcctttcctcagagggtatctgaacaagtgcaaagatctgcagagcaggcgacttgcctttttcaatgacattttcatccaggaaaggaggaagattttagagaagggggagcagatgacgaccaagtgtgccatagaccacatattggaggcggagaagaagggagaaataaacgagaaaaacgtggtgtacatagtggagaacataaacgtggcggcgatagagacgacactgtggtcgatggagtgggctcttgccgagctggtgaaccatccggaagtgcagcgcaaggtgagaagcgaggtggagagcatagtgggaagaggggcggcagtgaaggaagcggacatcgagaagcttccatacctgcaagcggtggtgaaggagacgctgaggctgcacacgcccattccgctgctggttccgcacatgaacttggacgatgcctcgctcggcgggttctccattccgagggagagcaaggtggttgtgaatgcgtggtggctggccaacaatccagagtggtgggatgatccctctgaattcaggcctgaaagatttatggaagaggagagggagactgaagcggctgtgggaggcaaagtcgacttccgtttccttccctttggcatgggtaggaggagttgcccaggcatcattctcgccctgcccgtgctcggcctcgttataggcagattgttgcagaatttcgagctcattccgccgcctgggagagagaagatcgacctgtctgaaaagggagggcaattcagtctccacattgccacccactccaccatccgcttccgccttatctgatgtcttaccacattat

SEQ ID NO: 37 - protein, 441 aa, Taxus baccata
  source 1..441: note = 3-N-debenzoyl-2-deoxytaxol-N-benzoyltransferase
MEKAGSTDFHVKKFDPVMVAPSLPSPKATVQLSVVDSLTICRGIFNTLLVFNAPDNISADPVKIIREALSKVLVYYFPLAGRLRSKEIGELEVECTGDGALFVEAMVEDTISVLRDLDDLNPSFQQLVFWHPLDTAIEDLHLVIVQVTRFTCGGIAVGVTLPHSVCDGRGAAQFVTALAEMARGEVKPSLEPIWNRELLNPEDPLHLQLNQFDSICPPPMLEELGQASFVINVDTIEYMKQCVMEECNEFCSSFEVVAALVWIARTKALQIPHTENVKLLFAMDLRKLFNPPLPNGYYGNAIGTAYAMDNVQDLLNGSLLRAIMIIKKAKADLKDNYSRSRVVTNPYSLDVNKKSDNILALSDWRRLGFYEADFGWGGPLNVSSLQRLENGLPMFSTFLYLLPAKNKSDGIKLLLSCMPPTTLKSFKIVMEAMIEKYVSKV

SEQ ID NO: 38 - RNA, 1326 nt, Taxus baccata
  source 1..1326: mol_type = mRNA; note = 3-N-debenzoyl-2-deoxytaxol-N-benzoyltransferase
atggagaaggcaggctcaacagacttccatgtaaagaaatttgatccagtcatggtagccccaagccttccatcgcccaaagctaccgtccagctctctgtcgttgatagcctaacaatctgcaggggaatttttaacacgttgttggttttcaatgcccctgacaacatttctgcagatcctgtaaaaataattagagaggctctctccaaggtgttggtgtattatttccctcttgctgggcggctcagaagtaaagaaattggggaacttgaagtggagtgcacaggggatggtgctctgtttgtggaagccatggtggaagacaccatttcagtcttacgagatctggatgacctcaatccatcatttcagcagttagttttttggcatccattggacactgctattgaggatcttcatcttgtgattgttcaggtaacacgttttacatgtgggggcattgccgttggagtgactttgccccatagtgtatgtgatggacgtggagcagcccagtttgttacagcactggcagagatggcgaggggagaggttaagccctcactagaaccaatatggaatagagaattgttgaaccctgaagaccctctacatctccagttaaatcaatttgattcgatatgcccacctccaatgctggaggaattgggtcaagcttcttttgttataaacgttgacaccatagaatatatgaagcaatgtgtcatggaggaatgtaatgaattttgttcgtcttttgaagtagtggcagcattggtttggatagcacggacaaaggctcttcaaattccacatactgagaatgtgaagcttctctttgcgatggatttgaggaaattatttaatcccccacttccaaatggatattatggtaatgccattggtactgcatatgcaatggataatgtccaagacctcttaaatggatctcttttgcgtgctataatgattataaaaaaagcaaaggctgatttaaaagataattattcgaggtcaagggtagttacaaacccatattcattagatgtgaacaagaaatccgacaacattcttgcattgagtgactggaggcggttgggattttatgaagccgattttgggtggggaggtccactgaatgtaagttccctgcaacggttggaaaatggattgcctatgtttagtacttttctatacctactacctgccaaaaacaagtctgatggaatcaagctgctactgtcttgtatgccaccaacaacattgaaatcatttaaaattgtaatggaagctatgatagagaaatatgtaagtaaagtgtga

SEQ ID NO: 39 - protein, 372 aa, Taxus baccata
  source 1..372: note = taxane 9 alpha-dioxygenase2
MSSNQKSFLPWNADVRDGLLEAGVLPYNGYTLDHVDGTKISASTFDNNGTRHTAADLLKYANPKNIVVLLNSTVSKILFNLESGNIKATGVDLTSDVDGLSYHVLINQLSHKSEVILSAGSIGSPQLLLLSGIGPSQQLRELNITVLLDLPSVGKGIQDPPLSSVIVESPKPLPFGITQVVGIVNDSQLYIEGLSFSQQNSTTNIQYSGLIGSKVPFPLSEGELRLSSINPQDTPSVRYNYLSDPFDLQECIVGVKIMANIIATDSIQKYKFAGNNNSSTFRFLGPVIPQNQSNNEDLAKFCRDTLASAFHFHGGCHIGSVIDKDHRVKGVDNLRVVDHSIFKDSQGTNPQATIMMLGRYIGVHIVQERMKL

SEQ ID NO: 40 - RNA, 1382 nt, Taxus baccata
  source 1..1382: mol_type = mRNA; note = taxane 9 alpha-dioxygenase2
ggtacgggtccagagttcttggcgggggagcaggccataaacggtgccttctacagcagggcgagcatggattttattaggaagatgaaatgggatgagaaacttgtaaatgagtcgtatgaatgggtggagaagttgaatgtcttcaaaccagaaaagctttctgccttggaatgctgatgtcagggatggtcttttggaagcaggagtgcttccctacaatggatatactttggatcatgtggatggcactaagatcagtgcttcaactttcgacaacaatggaacgagacatacagcggcagatcttctcaaatatgcgaacccgaaaaacattgtagttcttctcaattctaccgtcagcaaaatcctcttcaacttggaatcgggaaatataaaggctacgggtgtggatctcactagcgatgttgatggcctctcttatcatgtattaataaaccagttgtcacataagagtgaggtaattttgtcagcaggaagcataggcagccctcaacttctgctcttaagtggaattggtccatcacaacaactaagagaattaaatattactgtgcttttagatttaccttctgtagggaaagggattcaagatccacctctttcttcagtaattgttgaatcccctaaaccacttccatttggtataacacaggtagtgggcatagtaaatgactcacaactctacattgagggtcttagtttttcccagcagaatagtaccacaaatattcaatattctggacttattggtagtaaggtgccatttccgttatcagagggcgaacttcgacttagtagcataaatccccaagatacgccttcagtccgatacaactacctatctgacccttttgatcttcaagaatgtatagttggtgttaagataatggctaatattattgccacggattctatccagaagtataaatttgcaggaaataacaactctagcacatttcgattccttgggccagtaatacctcaaaatcaatcaaataatgaagacctagctaaattctgtagagatacactagcttcagcgtttcatttccatggaggttgtcatattggttcagtgattgacaaggaccatcgagtgaaaggtgtggataatctaagagtggtggatcattcaatttttaaagatagtcaagggactaatccacaagctactatcatgatgctcggaaggtatataggagtgcatattgtccaagagcgcatgaaactttgaagattctaagctccgagtgtcaataaagttattttcacacttttacacttttgtaatgacttgaaaatttgcaacgatgaaattcaataatactattgggagaaaagaaataattaccatttct

SEQ ID NO: 41 - protein, 526 aa, Taxus baccata
  source 1..526: note = taxane 9 alpha-dioxygenase3
MLAYFHHSFGGNDTNFGLSFMTADAALASGRSYDYIIVGGGTAGCPLAATLSQHFSVLVLERGGSPYGNPDIENRDRFGKPLREADNYTSIAQGFVTEDGLLLHRARVLGGATAINAGFYSRASLEYIRNMGWDEKLVNSSYEWVEKQNAFRPNKLSGWASAFKNALLQAQFLPYNGYTVDHVEGTKISASTFDNNGKRHTAADLLQKANPKNIVVLLNATASRILFNSTGGKLKASGVEFLSTVNGQSYKVLLSQFSGRSEVILSAGSLGSPQLLLLSGIGPSEHLKEFNIPVLLNLTSVGKDVQDNPGTTMRVESPIPLRISSPQVVAILNNSQIYVFSGSSVDQVPINGTSNSTRTRYSGSFFEKVAFPLSRGELRLRTKDPRDNPSVRYNYLSHPLDLQLCVQAVRVMSKVSETASIQQFTFQNSSSSPRGFRFIGTAMPDSDSDDKTVEKFCHEGLASHWHYHGGCNVGSVIDKSHRVNGVNGLRVVDCSTYIDIPGTNPQATTMMLGRYTGIKILQERLQ

SEQ ID NO: 42 - RNA, 1988 nt, Taxus baccata
  source 1..1988: mol_type = mRNA; note = taxane 9 alpha-dioxygenase3
taaacgcatttgatattgtaagtttagaacagaaggagaagtgggattcagtgaagattaaacgcatttgatattgaagtttagcagagaaggagaagcgggatctgtgaagatgaagatcatactgctgttatttcatgcttgcttattttcaccattcatttggaggcaacgacaccaacttcggattatccttcatgacagctgatgctgcgttggcgtccggaagatcatacgattacattatcgttggaggaggaacagccggttgtccccttgctgcaactctgtcccaacacttttctgttttggtattggagagaggaggctctccttacggaaatcccgacatcgagaaccgagaccgttttggaaagccgttgcgagaagcagataattacacatccatagctcagggatttgtgacggaagacggtttactgttgcacagagcaagagttttgggcggcgcaactgccatcaacgctggtttctacagcagagccagcttggaatacattcggaacatgggatgggatgaaaaactcgtcaacagttcgtacgagtgggtggagaaacagaatgccttcagacccaacaaactttctggatgggcatcggctttcaaaaatgcccttcttcaagctcaatttcttccttacaatggatatactgttgatcatgtggagggtaccaagattagtgcctccacgtttgataacaacgggaagagacacacagccgcagatcttctccagaaagccaaccctaaaaacattgttgttcttctcaacgctacagccagcagaatcctcttcaattccacaggaggtaaactgaaggcttctggagtagaattcctgagcactgttaatggccaatcctataaagtactactaagtcagttttcaggccgcagcgaggtaattttgtcggcaggaagcctgggaagccctcaacttcttctcctaagtggaattggcccttctgaacatttgaaagagttcaatattcctgtcctcttaaatttaacatccgtgggaaaagatgtgcaagataatcccggtacaaccatgagggtggaatcccccataccgcttcgaatctcaagcccgcaagtagtagccattctcaacaattcccaaatctatgtcttttctggcagctctgttgatcaagttcccattaatggcacatcaaattctacaaggacccgatattccggatcattttttgaaaaagtggcgtttcccctatccagaggagagctccgactgcgcaccaaagatcctcgagacaacccttcagttcgatacaactatttgtctcaccctctagatctgcagctgtgcgtgcaggctgtgagggtaatgtccaaggttagcgagacagcttctattcaacaatttacatttcagaatagttcaagcagccctagggggtttagattcattgggacagcgatgcctgacagcgattcggacgataaaacagtagaaaagttctgtcatgaaggacttgcttcccattggcactaccatggagggtgtaacgttggttctgtaattgacaaaagccatagagtgaacggggttaatggattaagggttgtggattgttcgacgtatatagatattcctggaacaaatccgcaagcaacaactatgatgctgggaaggtatactggaataaagattctgcaggagcgattacagtaaaatatggaaaaatcgtccctgaacaactcattgcatcgcgttgctgtttggtcaccaatctagtgtagaagattgattttcctgtaatttatatcttagctgcaattttttttaatattgttgtgagacacacctattatgaaatactttaaaaatcaattcctccaatccaaattaaaggcaaaatctctccatattgttatatatttgtgtatgtagatatttacatgtccttatatttttatatatatatatatatatatgtaataa

SEQ ID NO: 43 - protein, 540 aa, Taxus baccata
  source 1..540: note = taxane 9 alpha-dioxygenase4
MAILFLVISCLLMFSNNPKLHGSEAATSDIEYPYSFMTVDAEKAASRTYDYIIVGGGAAGCPLAATLSQHYSVLVVERGDSPYGNPDVETTGGFFKILLNADDYPYVAQRFVTEDGVQLVRGRVLGGGTAVNAAFYSRASQEYIRNMGWDEKLVNESFEWVEKLNAFEPDELTPWSSSLKNGLLEAGVLPYNGYTVEHLEGTKISASIFDNNGKRHTAADLLRYANPDNIVVLLNATVGRILFNQESGEINAVGVEFTSDVDGVFHNVSINQLSQRSEVILSAGTIGSNQLLLLSGIGPSQELKELNITVLLDLPFVGKGISDPPLASVNLESPKPLPSVSVQVAGILDDSQLYIEGLSYSIDNNATNRQYIGLIGSKVAFPLSRGELRINSTDPKVTPSVRYNYLSDPFDLEKCMLGVRVMANLTATKSFQEYKFTSSDNSSTFQFLGPALPQNQSNNEDLANFCRDTLGSFFHYHGGCHIGSVVDEKYRVNGVNNLRVVDGSIYKDSPGTNPQATTMMLGRYTGIRIIEEQNLYHSTS

SEQ ID NO: 44 - RNA, 1623 nt, Taxus baccata
  source 1..1623: mol_type = mRNA; note = taxane 9 alpha-dioxygenase4
atggcgattctattccttgtgatttcatgcctgttaatgtttagcaataatccgaagttacacggttcagaggcagcaacatcggatattgagtacccatattcgtttatgacagtagatgctgaaaaggcagcttcaagaacatatgattacattatcgttggaggaggtgcagcagggtgtcctttagcagcaactctgtcacagcattactctgttcttgttgtggagaggggagattctccttatggaaatcctgacgtcgagacgaccggtggttttttcaagattttgttgaatgcggatgattacccatatgtagctcaaagatttgtcacagaagatggagtacagttggtaaggggaagagtcctaggaggcggaacagctgtcaacgctgccttctacagcagggcgagccaggaatatattaggaatatgggatgggatgagaaacttgtaaacgagtcgtttgagtgggtggagaagttgaatgccttcgaaccagacgagcttaccccttggagttcttcgcttaaaaatggtcttctggaagctggagtgcttccctacaatggatatactgtggaacatttggagggcaccaagatcagtgcctcaatatttgataacaatggaaagagacatacagcagcagatcttctcagatatgcgaatccagataacattgtagttcttctcaatgctactgtcggcagaatcctcttcaatcaggaatcaggagagataaacgctgttggtgtagagttcacgagtgatgttgatggcgtctttcataatgtatcaattaatcaattgtcacaaaggagtgaggtgattttgtcagcaggaaccataggcagcaatcaacttcttctcttaagtggaattggtccatcacaagaactcaaagaattgaatattactgtgcttttagatttaccatttgtagggaaagggatttcagatccacctcttgcgagtgtcaatctagaatcccctaaacccttgccatctgtttcagtacaagttgcaggcatactagatgattcacaactctatattgagggtcttagttattctatagataataatgccacaaaccgtcaatacattggactaattggtagtaaggtagcatttcccttatccaggggtgagcttcgaattaatagcacagatcccaaagtcactccctcagttcgatacaactacctttctgacccttttgatctagaaaaatgcatgcttggtgtaagggtaatggctaatcttactgctaccaaatcttttcaagaatataaatttactagcagtgacaactctagcacatttcaattccttggacccgcattaccacaaaatcaatcaaacaatgaagaccttgccaacttctgtagagatacattaggttcattttttcattaccatggagggtgtcatattggttctgtggttgatgaaaaatatcgagtgaatggtgtcaataatctaagggtcgtggatggttcaatttacaaagacagcccagggactaatccacaagcaactaccatgatgcttggaaggtataccggaattcgtatcatcgaagagcagaatttgtatcattcaacatcatag

SEQ ID NO: 45 - protein, 802 aa, synthetic construct
  source 1..802: note = truncated taxadiene synthase 1
MSSSTGTSKVVSETSSTIVDDIPRLSANYHGDLWHHNVIQTLETPFRESSTYQERADELVVKIKDMFNALGDGDISPSAYDTAWVARVATISSDGSEKPRFPQALNWVFNNQLQDGSWGIESHFSLCDRLLNTTNSVIALSVWKTGHSQVEQGTEFIAENLRLLNEEDELSPDFEIIFPALLQKAKALGINLPYDLPFIKSLSTTREARLTDVSAAADNIPANMLNALEGLEEVIDWNKIMRFQSKDGSFLSSPASTACVLMNIGDEKCFTFLNNLLDKFGGCVPCMYSIDLLERLSLVDNIEHLGIGRHFKQEIKGALDYVYRHWSERGIGWGRDSLVPDLNTTALGLRTLRTHGYDVSSDVLNNFKDENGRFFSSAGQTHVELRSVVNLFRASDLAFPDEGVMDDARKFAEPYLRDALATKISTNTKLFKEIEYVVEYPWHMSIPRLEAGSYIDSYDDDYVWQRKTLYRMPSLSNSKCLELAKLDFNIVQSLHQEELKLLTRWWKESGMADINFTRHRVAEVYFSSATFEPEYSATRIAFTKIGCLQVLFDDMADIFATLDELKSFTEGVKRWDTSLLHEIPECMQTCFKVWFKLMEEVNNDVVKVQGRDMLAHIRKPWELYFNCYVQEREWLEAGYIPTFEEYLKTYAISVGLGPCTLQPILLMGELVKDDVVEKVHYPSNMFELVSLSWRLTNDTKTYQAEKARGQQASGIACYMKDNPGATEEDAIKHICRVVDRALKEASFEYFKPSNDIPMGCKSFIFNLRLCVQIFYKFIDGYGIANEEIKDYIRKVYIDPIQV

SEQ ID NO: 46 - RNA, 2409 nt, synthetic construct
  source 1..2409: mol_type = other RNA; note = truncated taxadiene synthase 1
atgagcagtagcactggcactagcaaggtggtttccgagacttccagtaccattgtggatgatatccctcgactctccgccaattatcatggcgatctgtggcaccacaatgttatacaaactctggagacaccatttcgtgagagttctacttaccaagaacgggcagatgagctggttgtgaaaattaaagatatgttcaatgcgctcggagacggagatatcagtccgtctgcatacgacactgcgtgggtggcgagggtggcgaccatttcctctgatggatctgagaagccacggtttcctcaggccctcaactgggttttcaacaaccagctccaggatggatcgtggggtatcgaatcgcactttagtttatgcgatcgattgcttaacacgaccaattctgttatcgccctctcggtttggaaaacagggcacagccaagtagaacaaggtactgagtttattgcagagaatctaagattactcaatgaggaagatgagctgtccccggatttcgaaataatctttcctgctctgctgcaaaaggcaaaagcgttggggatcaatcttccttacgatcttccatttatcaaatctttgtcgacaacacgggaagccaggcttacagatgtttctgcggcagcagacaatattccagccaacatgttgaatgcgttggagggtctcgaggaagttattgactggaacaagattatgaggtttcaaagtaaagatggatctttcctgagctcccctgcctccactgcctgtgtactgatgaatataggggacgaaaaatgtttcacttttctcaacaatctgctggacaaattcggcggctgcgtgccctgtatgtattccatcgatctgctggaacgcctttcgctggttgataacattgagcatctcggaatcggtcgccatttcaaacaagaaatcaaaggagctcttgattatgtctacagacattggagtgaaaggggcatcggttggggcagagacagcctcgttccagatctcaacacaacagccctcggcctgcgaactcttcgcacgcacggatacgatgtttcttcagatgttttgaataatttcaaagatgaaaacgggcggttcttctcctctgcgggccaaacccatgtcgaattgagaagcgtggtgaatcttttcagagcttccgaccttgcatttcctgacgaaggagttatggacgatgctagaaaatttgcagaaccatatcttagagacgcacttgcaacaaaaatctcaaccaatacaaaactattcaaagagattgagtacgtggtggagtacccttggcacatgagtatcccacgtctagaagccggaagttatattgattcatatgacgatgattatgtatggcagaggaagactctatacagaatgccatctttgagtaattcaaaatgtttagaattggcaaaattggacttcaatatcgtacaatctttgcatcaagaggagttgaagcttctaacaagatggtggaaggaatctggcatggcagatataaatttcactcgacaccgagtggcggaggtttatttttcatcagctacatttgaacccgaatattctgccactcgaattgccttcacaaaaattggttgtttacaagtcctttttgatgatatggctgacatctttgcaacactagatgaattgaaaagtttcactgagggagtaaagagatgggatacatctttgctacatgagattccagagtgtatgcaaacttgctttaaagtttggttcaaattgatggaagaagtaaataatgatgtggttaaggtacaaggacgtgacatgctcgctcacataagaaaaccctgggagttgtacttcaattgttatgtacaagaaagggagtggcttgaagctgggtatataccaacttttgaagagtacttaaagacttatgctatatcagtaggccttggaccgtgtaccctacaaccaatactactaatgggtgagcttgtgaaagatgatgttgttgagaaagtgcactatccctcaaatatgtttgagcttgtatccttgagctggcgactaacaaatgacaccaaaacatatcaggctgaaaaggctcgaggacaacaagcctcaggcatagcatgctatatgaaggataatccaggagcaactgaggaagatgccatcaagcacatatgtcgtgttgttgaccgagccttgaaagaagcaagctttgaatatttcaaaccatccaatgatatcccaatgggttgcaagtcctttatttttaaccttagattgtgtgtccaaatcttttacaagtttatagatgggtacggaatcgccaatgaggagattaaggattatataagaaaagtttatattgatccaattcaagtatga

SEQ ID NO: 47 - protein, 764 aa, synthetic construct
  source 1..764: note = truncated taxadiene synthase 2
MSGSPTKLATENANAVAESNLIPRLSANYHGDLWHHGVIQTLQTPYQESSSYQERAEELIVKIKDMFKAVEEGAISPSAYDTAWVARVPDGSEKPRFPQALNWLLHNQLQDGSWGLESHFMLSDRLLSTLNSVISLLVWKTGQQQVEQGTLFITENLKLLEGEDELPPDFEIIFPALLQKAKALGMSLPDHDLPFIKSLSVAREARLASYTDNNIPASMLNALEGLEEVIDWDKIMRFQMPCLYSIDLLERLSLVDNIEHLGIGRHFKQEIKVALDYVYRYWSERGIGLGRDSLIPDLNTTALGLRTLRAHGYNVSSEVLNNFKDENGRFFSSLGQTHVELRSMVNLLRASDLAFPDEPLMDDAKIFAEAYLRDALATRISTNTKLFKEIDYAVEYPWHMSIPRLEARSYIDVYDDDYTWQNKTLYSYNLCNRMSNLSNAYCLELAKLDFNIVQSLHQEELKLLTRWWKESGMADINFTRHRVAEVYFSSATFEPEYSSTRIAFTKIGCLQVLFDDMADIFATLDELRDFTEGVKRWDTSLIHKLPDCMQTCFRVWFNLMEEVNNDVSNVQGRDMLNHIRKPWELYFNCYVQEREWLDAGYIPTLEEYLKTYSISVGLGPCTLQPILLMGDIVKDDVVEKVHYPSNLFELVSLSWRLTNDTKTYQAEKARGQQASGIACYMKDNPGSTEEDAIKYICGVVDRALKEACFEYFKPADDVPMSCKSFIFNLRLCVQIFYKFIDGYGIANEEIKDYIRKVYIEPIQV

SEQ ID NO: 48 - RNA, 2295 nt, synthetic construct
  source 1..2295: mol_type = other RNA; note = truncated taxadiene synthase 2
atgagcggtagcccgaccaagttggctacggagaatgccaatgcagttgcagaatctaatttgatccctcgactctccgccaattatcatggcgatctgtggcaccatggcgtaatacaaacattacaaacaccttaccaagagagttcttcctaccaagaacgggcagaggagcttattgtgaaaattaaagatatgttcaaggcagttgaagagggagcaataagtccatccgcatacgacactgcctgggtcgcaagggtgcctgatggatctgagaagccacggtttccccaggccctcaactggcttctacacaaccagctccaagatggatcatggggtcttgaatcgcactttatgctgagcgatcgattgcttagcacactcaattctgttatctccctccttgtttggaaaacagggcagcagcaagtagaacaaggtactttgtttattacagagaatctaaaattactggagggggaagatgagttgcccccggactttgaaataatctttcctgctctgttgcaaaaggcaaaagcgctgggaatgagtcttcctgatcatgatcttccattcatcaaatctttgtcggtagcacgggaagcgaggcttgcaagttacacagacaacaatattccagccagcatgttgaatgcgttggagggtctggaggaagttattgattgggacaagattatgaggtttcaaatgccctgtttgtattcaatcgatctgcttgaacgcctttcgctggttgacaacatcgagcatctcggaatcggtcgacatttcaaacaagaaatcaaggtagctcttgattatgtctacagatattggagtgaaagaggcatcggtttgggtagagacagcctaattcctgatctgaacactacagccctcggcctccgaacccttcgggcccatggatacaatgtttcctcggaggttttgaataatttcaaagatgaaaacgggcgcttcttctcctctcttggccaaacacatgtagaattgagaagcatggtgaaccttttgagagcttccgacctcgcatttcccgacgaaccacttatggacgatgctaaaatctttgcagaagcatatcttagagacgcacttgcaacacgcatctcaaccaatacaaaattattcaaagagatcgactacgcggtagagtacccttggcacatgagtatcccacgtctcgaggcgagaagttatattgatgtatacgacgatgattatacatggcaaaataagactctatacagttacaatctgtgcaacagaatgtcaaacttgagtaacgcatattgcttagaattggcgaaattggacttcaatattgtgcaatctttgcatcaagaggagttgaagcttctaacaagatggtggaaagaatctggcatggcagatataaacttcactcgacaccgagtggcagaggtgtatttttcatcagctacgtttgaacccgaatattcttctaccagaatcgccttcaccaaaattggttgtttgcaagtcctgtttgacgacatggccgacatctttgcaacactagatgagttgagagatttcaccgagggagtaaagagatgggacacctctttgatacacaagctaccagactgtatgcaaacttgctttagagtttggtttaacttaatggaagaagtcaataacgacgtgtcaaacgtacaaggccgtgacatgctcaatcacataagaaaaccctgggagttgtacttcaattgttatgtacaagaaagagagtggctcgatgctgggtatataccgactctagaggagtacctaaagacctattctatatcagtaggccttggaccatgtactctacaaccaatactactaatgggcgatatcgtgaaagatgatgttgtcgagaaagtgcactatccctcaaatctatttgaacttgtatccttgagctggcgattaacaaatgacacaaaaacatatcaggctgagaaggctcgaggacaacaagcctcaggcatagcgtgttatatgaaggataatccaggatcgacagaggaagatgccatcaagtacatatgcggagttgttgatcgagccttgaaagaggcatgctttgaatatttcaagccagccgatgatgtcccaatgagttgcaagtcctttattttcaacctcagactgtgtgtccaaatattttacaagtttatagatgggtatggaattgccaacgaggagattaaggattatataagaaaagtttacattgaaccgattcaagtatga